European Patent Application EP 4 729 618 A1, published April 22, 2026. Title: ecombinant Vector for High-Expression of Gene. Applicant: CJ CheilJedang Corporation. The sequence listing filed with the application follows.

SEQUENCE LISTING (15 sequences)

SEQ ID NO: 1 - DNA, 1946 bp, synthetic construct
  misc_feature 1..1946: note = Site1_Contig 3, 2001468 (HindIII), SCH_00001433, from Schizochytrium sp.
  source 1..1946: mol_type = other DNA
agtgcacgaggcccgatctcataaccggcaatatcataaatttgatgtgcaagctctcgtccagtcttgctatccgggtcttcacaaatatacgatctaacaagcttttcatatgcttctctggttactttgggggcatgcagcccaccatcttcctccgatacctcctttgctcgcgatgcattatactttttagccccctcttcactactctgagattgagagctaagtcgtttcgcgtgttctgcttcctgttcagcaataaatgctgctagtgattcttcctcttcccttgcataccgcgtcatacgttcctcttctgtttcttcaccctgactacttttatcaagatcgccaggtgttgtgaaatcgtcatcgctagaatcggattgcacacttacaatatgtgaagtattaagaagcaactcactgtctcgttgaatagctgccgccccatgctgagcagcaagaccaatttgagacgtgtgcataaccaccggacgagacgaccgccgctttcttcctgatgttgtattaaacatgtcaagaatatctaaagacgaatctagttgggtttccccatcttcaattcgcgccatggtcacacgaatattaccttttcgacgtggatttgacataaaagtctttgtggaatttgatgatgcagaagatgaagaggagactgatgaagccatagacagaccgcgaccgctcagagtgtctggatgagcatgactgctgctttcaccttctataccggagtagcttgtagtactcagtgcatcaagcgctgcatgactgctactttcagcctctaatccgctatagctagcaatgctaagtccatcgggcgggacatagctattgctttcgccgtcaaatccaatgtagcttgtaatactaagcgcatctggagctacatgactgacgctgtcaccttcataaccgtgaccgctagcataactgctttcctcctcttctgttcgtgcaagcatatgaccaatattctgaaactccacatggccccttctagacgaaaagtcattcaatctggattccaggctcaatgactcgtgcgcatcaatgtgcgatgaggattgacttacctcgtcatatatttgtgagtttgctgtatcatccgcataatccgggtcatgctcactcgatgtagcaagtgcttcgtcatgatctgaaggaatgtcgtcttcaacttcagatccgtctgcctccctgcttgagatatcagggttcgagtctaggtcatctttgcctatcgaaggcgaattacgaggctctgaacttgtttcgacagatgcggtcggggtatcatcctgctccatagtctcttggtcaattctgctgatagtgctgtctccttcttgagactggccctgaatatcacttgattctgtactgccaaatgtagacaagttcagagaaggggttgaaatgttcagagatctaacagtcccgaagtgattcccatcgtttgaagatgactcagactcaactcttgagagaaatgtcccaacgccacttcccctaggttcttttgaaccagcgctttcgccgctagcggttgaccagtggtttaggaaggaagtctgctgatctgaagcagctaggaaaatgttggcttcatcttcatctttcgtcacctttccatcatcagggttcttaccaaggtggatgtctgccaagttaacttctgatccatcctggctagattgaactgtctctaaagtctctttcgcaattcctgacgtgtcttcaagttcttcataatcactttgctcgctagttgaaatattatctgccgagctcgcgtccgaattcaccattggatgttctgaaagagctcttttaatagaaatctcctcaggactacggtcagacagctcctgcgctgcctcagcaccatcatcattgacacatctaatgttgtt

SEQ ID NO: 2 - DNA, 2016 bp, synthetic construct
  misc_feature 1..2016: note = Site 2_Contig 3, 1116023 (HindIII), SCH_00001298, from Schizochytrium sp.
  source 1..2016: mol_type = other DNA
taggccttaggtagccagccatagctcgagcgtcgcgagaatccatctttcgatcaagaactaaggcaggaaaggaaatgaatgaaggcctcatgcgaatgtgcggtcatccgcggagtctcttgccgcggagcaagcaagcctcgcaggccttaagtggggtccatgggcggcgggcggcaacgactccgaaatgctttgtgaagaaagcaaacgcaggctagatgctagatgtggcgagaactccttcaggaccttgacgccgaggtctttctttctgcaacaaagattgatgtgataattctcaactctgacaagcgatgccgctctacttacttacctctggagttactacttactgcttctgtcgggactccaaagcattacatttccatccttggagactgtaatgtatccatgtaaatcgtgatcgaagttgacaagcaggccaaacaaagcacgagccgcaatgctgcacaacaaacaaacagatagatagatagatatcttgcagcctggggaccgctttggcaagcttttatggcttgaacaagacatgatcctgcgtttatctcaaagagccacgcgcaatctgcacaggctgcttaacctcgaagcagcgctgtcgttgagactaatcaatctctcgcaacgggagagctgctcgggaggttcttttcggatgtgtggctcaccttgcttgggggttcctgtaatatctgcttctcaattaacatttactaccacatgttggaaacaccctcacatctattaccagaaaaggaatttccgtccgcgataggttcacagaccgcgcaggtcgtagcacgcgcaggaaccactattttaaagactgcgcaactcggtcctgcctgaaaagaaatattttgtactcattaggaaatacgtagtcaattaatagcactaatttgtataggcctacctaacagtagtactatatgaatattttttaagaattgaggtagtcctggcagtagaccctggagttgatggagtcatcaccattctacttttgagattcgtctgcttttacctataggtagttcggtattgtcttttcgaaaatgataatgagaaaaacactgtcaggttcaacttagttgctaactctttgcatgacatgttgtgttttgtaatctattctgcgaactcgagacttgaactagcagccgagatagtgtgacaaacttcattgggaaggacgcaaggttatcaaatgtatagcgggaggattgatttgtgaatttgtttaccttagagaggctgccttttctttaggtaccactactaccacttgcaaaggaacttactccgagggacgatgagaggtgatgcgtggttggtagagggatttttgcgcctggcattgaaacatttcgcatcaggtggtaccttgtattgctgatatacaatggagtgattattttggcttgagtctttacccaagttcaaagactgatagtagttctatctgagagctgatctgccttgactcgaatttctacccaactagttagtgaaaactcatttgcgttaatgagtagttgccacgtagtacaggagcatgtagtatgcaaactttcaattcaaattaggggaaagttcctcggtgagagagtgattattacgaggaaccaaagttccacctgcttacaactgcacaaataagaagcacacggcgtcatactagttttgccgagttggtcaagagaattcattgtagactttccaacgatgttattagacaaaacactatttttcttctgcttcagcaacagagaaatgggtttgcttaacttccgtgcggtcttctgtcttggatgaataatcaaaatctacagcttataaaaattatttaagtgtacgcaaaatgtggtcttatccactttcatttacgttctgtgtactacgaataaataaattacagaattgaatttgggtatctactagagtcaaccacaacgaccacagtcaaggttgcagactttaacatat

SEQ ID NO: 3 - DNA, 1092 bp, synthetic construct
  misc_feature 1..1092: note = GFP coding gene
  source 1..1092: mol_type = other DNA
tccaaaggtgaagagctgttcactggcgtggttcccattctcgtcgaattggacggcgacgtgaacggacacaagttttctgtccgtggcgagggtgagggagacgccacaaatggcaagctcacattgaagttcatttgcactacaggcaaacttcctgttccgtggccgaccctcgtgactaccctcacctacggcgttcaatgcttctctcgttacccggatcatatgaagcgtcacgacttctttaagagtgctatgcccgaaggatacgttcaggagcgtaccattagctttaaggacgacggtacctacaagacccgcgccgaggtgaagttcgaaggcgacactcttgttaaccgcatcgaactcaagggcatcgactttaaagaggacggtaatattcttggccacaagctcgaatacaactttaactctcacaacgtttacatcactgccgacaagcaaaagaacggcattaaggctaactttaaaatccgtcataacgtggaggacggtagcgttcaactggctgatcattatcaacagaacacacccatcggcgacggtcccgtgcttctccccgacaatcattatctttccactcaatcggttttgtccaaggacccgaatgagaaacgtgaccacatggttcttttggagttcgtcacagccgctggcatcactcacggaatggacgaactctacaagggcggaggtagcgccaagttgaccagtgccgttccggtgctcaccgcgcgcgacgtcgccggagcggtcgagttctggaccgaccggctcgggttctcccgggacttcgtggaggacgacttcgccggtgtggtccgggacgacgtgaccctgttcatcagcgcggtccaggaccaggtggtgccggacaacaccctggcctgggtgtgggtgcgcggcctggacgagctgtacgccgagtggtcggaggtcgtgtccacgaacttccgggacgcctccgggccggccatgaccgagatcggcgagcagccgtgggggcgggagttcgccctgcgcgacccggccggcaactgcgtgcacttcgtggccgaggagcaggac

SEQ ID NO: 4 - DNA, 1000 bp, synthetic construct
  misc_feature 1..1000: note = 5'-homology arm_Site 1
  source 1..1000: mol_type = other DNA
agtgcacgaggcccgatctcataaccggcaatatcataaatttgatgtgcaagctctcgtccagtcttgctatccgggtcttcacaaatatacgatctaacaagcttttcatatgcttctctggttactttgggggcatgcagcccaccatcttcctccgatacctcctttgctcgcgatgcattatactttttagccccctcttcactactctgagattgagagctaagtcgtttcgcgtgttctgcttcctgttcagcaataaatgctgctagtgattcttcctcttcccttgcataccgcgtcatacgttcctcttctgtttcttcaccctgactacttttatcaagatcgccaggtgttgtgaaatcgtcatcgctagaatcggattgcacacttacaatatgtgaagtattaagaagcaactcactgtctcgttgaatagctgccgccccatgctgagcagcaagaccaatttgagacgtgtgcataaccaccggacgagacgaccgccgctttcttcctgatgttgtattaaacatgtcaagaatatctaaagacgaatctagttgggtttccccatcttcaattcgcgccatggtcacacgaatattaccttttcgacgtggatttgacataaaagtctttgtggaatttgatgatgcagaagatgaagaggagactgatgaagccatagacagaccgcgaccgctcagagtgtctggatgagcatgactgctgctttcaccttctataccggagtagcttgtagtactcagtgcatcaagcgctgcatgactgctactttcagcctctaatccgctatagctagcaatgctaagtccatcgggcgggacatagctattgctttcgccgtcaaatccaatgtagcttgtaatactaagcgcatctggagctacatgactgacgctgtcaccttcataaccgtgaccgctagcataactgctttcctcctcttctgttcgtgcaagcatatgac

SEQ ID NO: 5 - DNA, 946 bp, synthetic construct
  misc_feature 1..946: note = 3'-homology arm_Site 1
  source 1..946: mol_type = other DNA
caatattctgaaactccacatggccccttctagacgaaaagtcattcaatctggattccaggctcaatgactcgtgcgcatcaatgtgcgatgaggattgacttacctcgtcatatatttgtgagtttgctgtatcatccgcataatccgggtcatgctcactcgatgtagcaagtgcttcgtcatgatctgaaggaatgtcgtcttcaacttcagatccgtctgcctccctgcttgagatatcagggttcgagtctaggtcatctttgcctatcgaaggcgaattacgaggctctgaacttgtttcgacagatgcggtcggggtatcatcctgctccatagtctcttggtcaattctgctgatagtgctgtctccttcttgagactggccctgaatatcacttgattctgtactgccaaatgtagacaagttcagagaaggggttgaaatgttcagagatctaacagtcccgaagtgattcccatcgtttgaagatgactcagactcaactcttgagagaaatgtcccaacgccacttcccctaggttcttttgaaccagcgctttcgccgctagcggttgaccagtggtttaggaaggaagtctgctgatctgaagcagctaggaaaatgttggcttcatcttcatctttcgtcacctttccatcatcagggttcttaccaaggtggatgtctgccaagttaacttctgatccatcctggctagattgaactgtctctaaagtctctttcgcaattcctgacgtgtcttcaagttcttcataatcactttgctcgctagttgaaatattatctgccgagctcgcgtccgaattcaccattggatgttctgaaagagctcttttaatagaaatctcctcaggactacggtcagacagctcctgcgctgcctcagcaccatcatcattgacacatctaatgttgtt

SEQ ID NO: 6 - DNA, 986 bp, synthetic construct
  misc_feature 1..986: note = 5'-homology arm_Site 2
  source 1..986: mol_type = other DNA
taggccttaggtagccagccatagctcgagcgtcgcgagaatccatctttcgatcaagaactaaggcaggaaaggaaatgaatgaaggcctcatgcgaatgtgcggtcatccgcggagtctcttgccgcggagcaagcaagcctcgcaggccttaagtggggtccatgggcggcgggcggcaacgactccgaaatgctttgtgaagaaagcaaacgcaggctagatgctagatgtggcgagaactccttcaggaccttgacgccgaggtctttctttctgcaacaaagattgatgtgataattctcaactctgacaagcgatgccgctctacttacttacctctggagttactacttactgcttctgtcgggactccaaagcattacatttccatccttggagactgtaatgtatccatgtaaatcgtgatcgaagttgacaagcaggccaaacaaagcacgagccgcaatgctgcacaacaaacaaacagatagatagatagatatcttgcagcctggggaccgctttggcaagcttttatggcttgaacaagacatgatcctgcgtttatctcaaagagccacgcgcaatctgcacaggctgcttaacctcgaagcagcgctgtcgttgagactaatcaatctctcgcaacgggagagctgctcgggaggttcttttcggatgtgtggctcaccttgcttgggggttcctgtaatatctgcttctcaattaacatttactaccacatgttggaaacaccctcacatctattaccagaaaaggaatttccgtccgcgataggttcacagaccgcgcaggtcgtagcacgcgcaggaaccactattttaaagactgcgcaactcggtcctgcctgaaaagaaatattttgtactcattaggaaatacgtagtcaattaatagcactaatttgtataggcctacctaacagtagtactatatgaatattttttaagaattgaggtag

SEQ ID NO: 7 - DNA, 1030 bp, synthetic construct
  misc_feature 1..1030: note = 3'-homology arm_Site 2
  source 1..1030: mol_type = other DNA
tcctggcagtagaccctggagttgatggagtcatcaccattctacttttgagattcgtctgcttttacctataggtagttcggtattgtcttttcgaaaatgataatgagaaaaacactgtcaggttcaacttagttgctaactctttgcatgacatgttgtgttttgtaatctattctgcgaactcgagacttgaactagcagccgagatagtgtgacaaacttcattgggaaggacgcaaggttatcaaatgtatagcgggaggattgatttgtgaatttgtttaccttagagaggctgccttttctttaggtaccactactaccacttgcaaaggaacttactccgagggacgatgagaggtgatgcgtggttggtagagggatttttgcgcctggcattgaaacatttcgcatcaggtggtaccttgtattgctgatatacaatggagtgattattttggcttgagtctttacccaagttcaaagactgatagtagttctatctgagagctgatctgccttgactcgaatttctacccaactagttagtgaaaactcatttgcgttaatgagtagttgccacgtagtacaggagcatgtagtatgcaaactttcaattcaaattaggggaaagttcctcggtgagagagtgattattacgaggaaccaaagttccacctgcttacaactgcacaaataagaagcacacggcgtcatactagttttgccgagttggtcaagagaattcattgtagactttccaacgatgttattagacaaaacactatttttcttctgcttcagcaacagagaaatgggtttgcttaacttccgtgcggtcttctgtcttggatgaataatcaaaatctacagcttataaaaattatttaagtgtacgcaaaatgtggtcttatccactttcatttacgttctgtgtactacgaataaataaattacagaattgaatttgggtatctactagagtcaaccacaacgaccacagtcaaggttgcagactttaacatat

SEQ ID NO: 8 - DNA, 48 bp, synthetic construct
  misc_feature 1..48: note = Forward primer
  source 1..48: mol_type = other DNA
cctcctcttctgttcgtgcaagcatatgacggtacccttgatcttgtg

SEQ ID NO: 9 - DNA, 42 bp, synthetic construct
  misc_feature 1..42: note = Reverse primer
  source 1..42: mol_type = other DNA
aggggccatgtggagtttcagaatattggcatgccttgaagc

SEQ ID NO: 10 - DNA, 45 bp, synthetic construct
  misc_feature 1..45: note = Forward primer
  source 1..45: mol_type = other DNA
atcatcattgacacatctaatgttgttaagcttggcgtaatcatg

SEQ ID NO: 11 - DNA, 45 bp, synthetic construct
  misc_feature 1..45: note = Reverse primer
  source 1..45: mol_type = other DNA
ccggttatgagatcgggcctcgtgcactgagctcgaattcactgg

SEQ ID NO: 12 - DNA, 27 bp, synthetic construct
  misc_feature 1..27: note = Forward primer_Site 1
  source 1..27: mol_type = other DNA
ttccttctgaagaagggtcgttggtct

SEQ ID NO: 13 - DNA, 20 bp, synthetic construct
  misc_feature 1..20: note = Reverse primer_Site 1
  source 1..20: mol_type = other DNA
ccaggaaaggacttgagatg

SEQ ID NO: 14 - DNA, 18 bp, synthetic construct
  misc_feature 1..18: note = Forward primer_Site 2
  source 1..18: mol_type = other DNA
gaaaaggacttgtgcctc

SEQ ID NO: 15 - DNA, 20 bp, synthetic construct
  misc_feature 1..20: note = Reverse primer_Site 2
  source 1..20: mol_type = other DNA
ccaggaaaggacttgagatg